European Patent Specification EP 3 559 239 B1, published September 25, 2024. Title: Oligomeric vaccines from plants by S-Tag-S-Protein fusions. Applicant: Leibniz-Institut für Pflanzengenetik und Kulturpflanzenforschung (IPK). The sequence listing filed with the application follows.

SEQUENCE LISTING (37 sequences)

SEQ ID NO: 1 - protein, 506 aa, Avian influenza virus
DQICIGYHANNSTEQVDTIMEKNVTVTHAQDILEKTHNGKLCDLDGVKPLILRDCSVAGWLLGNPMCDEFINVPEWSYIVEKANPVNDLCYPGDFNDYEELKHLLSRINHFEKIQIIPKSSWPSHEASLGVSSACPYQGKSSFFRNVVWLIKKNSTYPTIKRSYNNTNQEDLLVLWGIHHPNDAAEQTKLYQNPTTYISVGTSTLNQRLVPRIATRSKVNGQSGRMEFFWTILKPNDAINFESNGNFIAPEYAYKIVKKGDSTIMKSELEYGNCNTKCQTPMGAINSSMPFHNIHPLTIGECPKYVKSNRLVLATGLRNSPQRERRGLFGAIAGFIEGGWQGMVDGWYGYHHSNEQGSGYAADKESTQKAIDGVTNKVNSIIDKMNTQFEAVGREFNNLERRIENLNKKMEDGFLDVWTYNAELLVLMENERTLDFHDSNVKNLYDKVRLQLRDNAKELGNGCFEFYHKCDNECMESVRNGTYDYPQYSEEAKLKREEISGVKLEG

SEQ ID NO: 2 - protein, 15 aa, Homo sapiens
KESRAKKFQRQHMDS

SEQ ID NO: 3 - protein, 15 aa, Bos taurus
KETAAAKFERQHMDS

SEQ ID NO: 4 - protein, 15 aa, Ovis aries
KESAAAKFERQHMDS

SEQ ID NO: 5 - protein, 15 aa, Capra hircus
KESAAAKFERQHMDS

SEQ ID NO: 6 - protein, 15 aa, Sus scrofa
KESPAKKFQRQHMDP

SEQ ID NO: 7 - protein, 15 aa, Equus caballus
KESPAMKFERQHMDS

SEQ ID NO: 8 - protein, 15 aa, Capreolus capreolus
KESAAAKFERQHMDP

SEQ ID NO: 9 - protein, 113 aa, Homo sapiens
DSSPSSSSTYCNQMMRRRNMTQGRCKPVNTFVHEPLVDVQNVCFQEKVTCKNGQGNCYKSNSSMHITDCRLTNGSRYPNCAYRTSPKERHIIVACEGSPYVPVHFDASVEDST

SEQ ID NO: 10 - protein, 109 aa, Bos taurus
STSAASSSNYCNQMMKSRNLTKDRCKPVNTFVHESLADVQAVCSQKNVACKNGQTNCYQSYSTMSITDCRETGSSKYPNCAYKTTQANKHIIVACEGNPYVPVHFDASV

SEQ ID NO: 11 - protein, 109 aa, Ovis aries
STSSASSSNYCNQMMKSRNLTQDRCKPVNTFVHESLADVQAVCSQKNVACKNGQTNCYQSYSTMSITDCRETGSSKYPNCAYKTTQAEKHIIVACEGNPYVPVHFDASV

SEQ ID NO: 12 - protein, 109 aa, Capra hircus; identical to SEQ ID NO: 11

SEQ ID NO: 13 - protein, 109 aa, Sus scrofa
DSSSSNSSNYCNLMMSRRNMTQGRCKPVNTFVHESLADVQAVCSQINVNCKNGQTNCYQSNSTMHITDCRQTGSSKYPNCAYKASQEQKHIIVACEGNPPVPVHFDASV

SEQ ID NO: 14 - protein, 113 aa, Equus caballus
GSTSSSNPTYCNQMMKRRNMTQGWCKPVNTFVHEPLADVQAICLQKNITCKNGQSNCYQSSSSMHITDCRLTSGSKYPNCAYQTSQKERHIIVACEGNPYVPVHFDASVEVST

SEQ ID NO: 15 - protein, 109 aa, Capreolus capreolus
SPSSASSSNYCNQMMQSRNLTQDRCKPVNTFVHESLADVQAVCFQKNVICKNGQSNCYQSNSAMHITDCRESGNSKYPNCVYKTTQAEKHIIVACEGNPYVPVHFDASV

SEQ ID NO: 16 - protein, 19 aa, Homo sapiens
KPTLYNVSLVMSDTAGTCY

SEQ ID NO: 17 - protein, 19 aa, Mus musculus
KPTLYNVSLIMSDTGGTCY

SEQ ID NO: 18 - protein, 19 aa, Gorilla gorilla
KPTLYNVSLVMSDTAGTCY

SEQ ID NO: 19 - protein, 19 aa, Macaca mulatta
KPTLYNVSLVMSDTAGTCY

SEQ ID NO: 20 - protein, 19 aa, Canis familiaris
KPTLYNVSLVLSDTAGZCY

SEQ ID NO: 21 - protein, 19 aa, Ailuropoda melanoleuca
KPTLYNVSLVLSDTASTCY

SEQ ID NO: 22 - protein, 19 aa, Oryctolagus cuniculus
KPTLYNVSLIMSDTASTCY

SEQ ID NO: 23 - protein, 170 aa, Artificial Sequence
  S-protein-pII fusion protein
GSHHHHHHGSSSSNYCNQMMKSRNLTKDRCKPVNTFVHESLADVQAVCSQKNVACKNGQTNCYQSYSTMSITDCRETGSSKYPNCAYKTTQANKHIIVACEGNPYVPVHFDASVGPKRMKQIEDKIEEILSKIYHIENEIARIKKLIGERAAAEQKLISEEDLNGSKDEL

SEQ ID NO: 24 - protein, 177 aa, Artificial Sequence
  S-protein-GCN4 fusion protein
SHHHHHHGSSSSNYCNQMMKSRNLTKDRCKPVNTFVHESLADVQAVCSQKNVACKNGQTNCYQSYSTMSITDCRETGSSKYPNCAYKTTQANKHIIVACEGNPYVPVHFDASVASGGGSGGGSGGGSRMKQLEDKVEELLSKNYHLENEVARLKKLVAAAEQKLISEEDLNGSKDEL

SEQ ID NO: 25 - protein, 147 aa, Artificial Sequence
  S-protein-tail piece fusion protein
GSSSSNYCNQMMKSRNLTKDRCKPVNTFVHESLADVQAVCSQKNVACKNGQTNCYQSYSTMSITDCRETGSSKYPNCAYKTTQANKHIIVACEGNPYVPVHFDASVASKPTLYNVSLIMSDTGGTCYAAAEQKLISEEDLNGSKDEL

SEQ ID NO: 26 - protein, 594 aa, Artificial Sequence
  H5-S-Tag fusion protein
GSDQICIGYHANNSTEQVDTIMEKNVTVTHAQDILEKTHNGKLCDLDGVKPLILRDCSVAGWLLGNPMCDEFINVPEWSYIVEKANPVNDLCYPGDFNDYEELKHLLSRINHFEKIQIIPKSSWPSHEASLGVSSACPYQGKSSFFRNVVWLIKKNSTYPTIKRSYNNTNQEDLLVLWGIHHPNDAAEQTKLYQNPTTYISVGTSTLNQRLVPRIATRSKVNGQSGRMEFFWTILKPNDAINFESNGNFIAPEYAYKIVKKGDSTIMKSELEYGNCNTKCQTPMGAINSSMPFHNIHPLTIGECPKYVKSNRLVLATGLRNSPQRERRGLFGAIAGFIEGGWQGMVDGWYGYHHSNEQGSGYAADKESTQKAIDGVTNKVNSIIDKMNTQFEAVGREFNNLERRIENLNKKMEDGFLDVWTYNAELLVLMENERTLDFHDSNVKNLYDKVRLQLRDNAKELGNGCFEFYHKCDNECMESVRNGTYDYPQYSEEAKLKREEISGVKLEGPKRMKQIEDKIEEILSKIYHIENEIARIKKLIGERGGGGSASKETAAAKFERQHMDSAAAHHHHHHLAAEQKLISEEDLNGSKDEL

SEQ ID NO: 27 - protein, 33 aa, Artificial Sequence
  Trimerization domain
RMKQIEDKIEEILSKIYHIENEIARIKKLIGER

SEQ ID NO: 28 - DNA, 8074 bp, Artificial Sequence
  pCB301_H5-S-Tag
cgctcaccgggctggttgccctcgccgctgggctggcggccgtctatggccctgcaaacgcgccagaaacgccgtcgaagccgtgtgcgagacaccgcggccgccggcgttgtggatacctcgcggaaaacttggccctcactgacagatgaggggcggacgttgacacttgaggggccgactcacccggcgcggcgttgacagatgaggggcaggctcgatttcggccggcgacgtggagctggccagcctcgcaaatcggcgaaaacgcctgattttacgcgagtttcccacagatgatgtggacaagcctggggataagtgccctgcggtattgacacttgaggggcgcgactactgacagatgaggggcgcgatccttgacacttgaggggcagagtgctgacagatgaggggcgcacctattgacatttgaggggctgtccacaggcagaaaatccagcatttgcaagggtttccgcccgtttttcggccaccgctaacctgtcttttaacctgcttttaaaccaatatttataaaccttgtttttaaccagggctgcgccctgtgcgcgtgaccgcgcacgccgaaggggggtgcccccccttctcgaaccctcccggcccgctctcgagttggcagcatcacccataattgtggtttcaaaatcggctccgtcgatactatgttatacgccaactttgaaaacaactttgaaaaagctgttttctggtatttaaggttttagaatgcaaggaacagtgaattggagttcgtcttgttataattagcttcttggggtatctttaaatactgtagaaaagaggaaggaaataataaatggctaaaatgagaatatcaccggaattgaaaaaactgatcgaaaaataccgctgcgtaaaagatacggaaggaatgtctcctgctaaggtatataagctggtgggagaaaatgaaaacctatatttaaaaatgacggacagccggtataaagggaccacctatgatgtggaacgggaaaaggacatgatgctatggctggaaggaaagctgcctgttccaaaggtcctgcactttgaacggcatgatggctggagcaatctgctcatgagtgaggccgatggcgtcctttgctcggaagagtatgaagatgaacaaagccctgaaaagattatcgagctgtatgcggagtgcatcaggctctttcactccatcgacatatcggattgtccctatacgaatagcttagacagccgcttagccgaattggattacttactgaataacgatctggccgatgtggattgcgaaaactgggaagaagacactccatttaaagatccgcgcgagctgtatgattttttaaagacggaaaagcccgaagaggaacttgtcttttcccacggcgacctgggagacagcaacatctttgtgaaagatggcaaagtaagtggctttattgatcttgggagaagcggcagggcggacaagtggtatgacattgccttctgcgtccggtcgatcagggaggatatcggggaagaacagtatgtcgagctattttttgacttactggggatcaagcctgattgggagaaaataaaatattatattttactggatgaattgttttagtacctagatgtggcgcaacgatgccggcgacaagcaggagcgcaccgacttcttccgcatcaagtgttttggctctcaggccgaggcccacggcaagtatttgggcaaggggtcgctggtattcgtgcagggcaagattcggaataccaagtacgagaaggacggccagacggtctacgggaccgacttcattgccgataaggtggattatctggacaccaaggcaccaggcgggtcaaatcaggaataagggcacattgccccggcgtgagtcggggcaatcccgcaaggagggtgaatgaatcggacgtttgaccggaaggcatacaggcaagaactgatcgacgcggggttttccgccgaggatgccgaaaccatcgcaagccgcaccgtcatgcgtgcgccccgcgaaaccttccagtccgtcggctcgatggtccagcaagctacggccaagatcgagcgcgacagcgtgcaactggctccccctgccctgcccgcgccatcggccgccgtggagcgttcgcgtcgtctcgaacaggaggcggcaggtttggcgaagtcgatgaccatcgacacgcgaggaactatgacgaccaagaagcgaaaaaccgccggcgaggacctggcaaaacaggtcagcgaggccaagcaggccgcgttgctgaaacacacgaagcagcagatcaaggaaatgcagctttccttgttcgatattgcgccgtggccggacacgatgcgagcgatgccaaacgacacggcccgctctgccctgttcaccacgcgcaacaagaaaatcccgcgcgaggcgctgcaaaacaaggtcattttccacgtcaacaaggacgtgaagatcacctacaccggcgtcgagctgcgggccgacgatgacgaactggtgtggcagcaggtgttggagtacgcgaagcgcacccctatcggcgagccgatcaccttcacgttctacgagctttgccaggacctgggctggtcgatcaatggccggtattacacgaaggccgaggaatgcctgtcgcgcctacaggcgacggcgatgggcttcacgtccgaccgcgttgggcacctggaatcggtgtcgctgctgcaccgcttccgcgtcctggaccgtggcaagaaaacgtcccgttgccaggtcctgatcgacgaggaaatcgtcgtgctgtttgctggcgaccactacacgaaattcatatgggagaagtaccgcaagctgtcgccgacggcccgacggatgttcgactatttcagctcgcaccgggagccgtacccgctcaagctggaaaccttccgcctcatgtgcggatcggattccacccgcgtgaagaagtggcgcgagcaggtcggcgaagcctgcgaagagttgcgaggcagcggcctggtggaacacgcctgggtcaatgatgacctggtgcattgcaaacgctagggccttgtggggtcagttccggctgggggttcagccagcgctttactgagatctggggaaccctgtggttggcatgcacatacaaatggacgaacggataaaccttttcacgcccttttaaatatccgattattctaataaacgctcttttctcttaggtttacccgccaatatatcctgtcaaacactgatagtttaaactgaaggcgggaaacgacaatctgatcatgagcggagaattaagggagtcacgttatgacccccgccgatgacgcgggacaagccgttttacgtttggaactgacagaaccgcaacgttgaaggagccactcagccgcgggtttctggagtttaatgagctaagcacatacgtcagaaaccattattgcgcgttcaaaagtcgcctaaggtcactatcagctagcaaatatttcttgtcaaaaatgctccactgacgttccataaattcccctcggtatccaattagagtctcatattcactctcaatccaaataatctgcaccggatctggatcgtttcgcatgattgaacaagatggattgcacgcaggttctccggccgcttgggtggagaggctattcggctatgactgggcacaacagacaatcggctgctctgatgccgccgtgttccggctgtcagcgcaggggcgcccggttctttttgtcaagaccgacctgtccggtgccctgaatgaactgcaggacgaggcagcgcggctatcgtggctggccacgacgggcgttccttgcgcagctgtgctcgacgttgtcactgaagcgggaagggactggctgctattgggcgaagtgccggggcaggatctcctgtcatctcaccttgctcctgccgagaaagtatccatcatggctgatgcaatgcggcggctgcatacgcttgatccggctacctgcccattcgaccaccaagcgaaacatcgcatcgagcgagcacgtactcggatggaagccggtcttgtcgatcaggatgatctggacgaagagcatcaggggctcgcgccagccgaactgttcgccaggctcaaggcgcgcatgcccgacggcgatgatctcgtcgtgacccatggcgatgcctgcttgccgaatatcatggtggaaaatggccgcttttctggattcatcgactgtggccggctgggtgtggcggaccgctatcaggacatagcgttggctacccgtgatattgctgaagagcttggcggcgaatgggctgaccgcttcctcgtgctttacggtatcgccgctcccgattcgcagcgcatcgccttctatcgccttcttgacgagttcttctgagcgggactctggggttcgaaatgaccgaccaagcgacgcccaacctgccatcacgagatttcgattccaccgccgccttctatgaaaggttgggcttcggaatcgttttccgggacgccggctggatgatcctccagcgcggggatctcatgctggagttcttcgcccacgggatctctgcggaacaggcggtcgaaggtgccgatatcattacgacagcaacggccgacaagcacaacgccacgatcctgagcgacaatatgatcgggcccggcgtccacatcaacggcgtcggcggcgactgcccaggcaagaccgagatgcaccgcgatatcttgctgcgttcggatattttcgtggagttcccgccacagacccggatgatccccgatcgttcaaacatttggcaataaagtttcttaagattgaatcctgttgccggtcttgcgatgattatcatataatttctgttgaattacgttaagcatgtaataattaacatgtaatgcatgacgttatttatgagatgggtttttatgattagagtcccgcaattatacatttaatacgcgatagaaaacaaaatatagcgcgcaaactaggataaattatcgcgcgcggtgtcatctatgttactagatcgggccaatacgcaaaccgcctctccccgcgcgttggccgattcattaatgcagctggcacgacaggtttcccgactggaaagcgggcagtgagcgcaacgcaattaatgtgagttagctcactcattaggcaccccaggctttacactttatgcttccggctcgtatgttgtgtggaattgtgagcggataacaatttcacacaggaaacagctatgaccatgattacgccaagcttgcatgcctgcaggtcactggattttggttttaggaattagaaattttattgatagaagtattttacaaatacaaatacatactaagggtttcttatatgctcaacacatgagcgaaaccctataagaaccctaattcccttatctgggaactactcacacattattctggagaaaatagagagagatagatttgtagagagagactggtgatttttgcggactctatcgacggatcgggctagagttcgtctttggaaccattcagatcctcttctgagatgagtttttgttctgcggccaaatggtgatggtggtgatgcgcggccgcggaatccatatgctgtctttcgaacttagctgctgctgtctctttgctagctgaaccacctccacctctttctccaataagtttcttgatacgagcgatctcgttctcgatatgataaatcttggaaagaatttcctcgatcttatcctcgatctgcttcattctcttgggcccctccaatttcacccctgaaatttcttcccgtttcaatttggcctcttcagaatactggggataatcatatgtgccattcctcacgctctccatgcactcattatcgcatttgtgataaaactcaaaacagccattcccaagctctttggcattatccctaagctgaagcctgactttgtcgtaaagatttttcacattgctatcgtgaaagtccaaagtacgctcattttccataagcaccaacaattcagcattatatgtccacacatcgagaaacccgtcctccattttcttattgagattttcaattcgacgttcaagattattgaattccctgccgactgcttcaaactgagtattcattttatcaataatagaattcactttgttagtgaccccatcaatagctttctgagttgattctttatcagcagcataacctgaaccctgttcatttgagtgatgataaccataccaaccatcaaccataccctgccaaccaccttcgataaaaccagcaatagcaccaaacaaacctcgacgttccctctgcgggctatttcgtaaaccagtagcgagaaccaaacgattagacttcacatacttcggacattctccaatggtcagggggtgaatattatgaaaaggcatgcttgaattaatagctcccataggggtttggcacttggtattacaattaccgtactccagctcgcttttcataatggttgagtcgcctttcttgactatcttgtaggcgtactcaggagcaatgaaattcccattggactcaaaattaattgcgtcattaggtttgagtatggtccaaaagaattccattcttccgctttgaccattaaccttacttctcgtagcaattcttggaacaagtctttggttgagagtggatgttccaacggatatgtatgtagttgggttttgatagagctttgtttgttctgctgcatcgtttggatgatgaattccccatagaacaagcagatcctcttggttcgtgttgttgtaactcctctttatggttgggtatgtggagttcttctttatcaaccacacaacgtttctgaagaatgaagattttccttgatatggacatgcagaactaactccaagagatgcttcatgactaggccaagaggacttcggtatgatctgaatcttctcgaagtggttaattctagatagcagatgcttaagctcttcgtaatcgttgaaatctccagggtaacacaaatcgttaactgggtttgccttttcaacgatgtaactccattctggaacgttgataaactcatcacacataggatttcctaacaaccatccagcaacggaacaatctctaaggatcaaaggcttaactccatctaggtcacatagctttccgttatgagtcttctcaaggatatcttgtgcatgtgtaaccgttacgttcttctccatgattgtgtctacttgctctgtactgttattagcatggtaaccgatgcagatttggtcggatcctgctaaacatgtgcttgtaaagagaagcaaggaaagtgaaagcaaagatagaaaaggtttggaagccatggttcccggccgggtcagatcctctagagtcgatcgaggtcctctccaaatgaaatgaacttccttatatagaggaagggtcttgcgaaggatagtgggattgtgcgtcatcccttacgtcagtggagatatcacatcaatccacttgctttgaagacgtggttggaacgtcttctttttccacgatgttcctcgtgggtgggggtccatctttgggaccactgtcggtagaggcattcttgaacgatagcctttcctttatcgcaatgatggcatttgtagaagccatcttccttttctactgtcctttcgatgaagtgacagatagctgggcaatggaatccgaggaggtttcccgatattaccctttgttgaaaagtctcaatagccctctggtcttctgagactgtatctttgatattcttggagtagacgagagtgtcgtgctccaccatgttgacctgcaggcatgcaagcttatcgataccgtcgacctcgagggggggcccggtaccaaaaccaccccagtacattaaaaacgtccgcaatgtgttattaagttgtctaagcgtcaatttgtttacaccacaatatatcctgccaccagccagccaacagctccccgaccggcagctcggcacaaaatcaccactcgatacaggcagcccatcagtccactaga

SEQ ID NO: 29 - DNA, 6733 bp, Artificial Sequence
  pCB_S-protein-tail piece
cgctcaccgggctggttgccctcgccgctgggctggcggccgtctatggccctgcaaacgcgccagaaacgccgtcgaagccgtgtgcgagacaccgcggccgccggcgttgtggatacctcgcggaaaacttggccctcactgacagatgaggggcggacgttgacacttgaggggccgactcacccggcgcggcgttgacagatgaggggcaggctcgatttcggccggcgacgtggagctggccagcctcgcaaatcggcgaaaacgcctgattttacgcgagtttcccacagatgatgtggacaagcctggggataagtgccctgcggtattgacacttgaggggcgcgactactgacagatgaggggcgcgatccttgacacttgaggggcagagtgctgacagatgaggggcgcacctattgacatttgaggggctgtccacaggcagaaaatccagcatttgcaagggtttccgcccgtttttcggccaccgctaacctgtcttttaacctgcttttaaaccaatatttataaaccttgtttttaaccagggctgcgccctgtgcgcgtgaccgcgcacgccgaaggggggtgcccccccttctcgaaccctcccggcccgctctcgagttggcagcatcacccataattgtggtttcaaaatcggctccgtcgatactatgttatacgccaactttgaaaacaactttgaaaaagctgttttctggtatttaaggttttagaatgcaaggaacagtgaattggagttcgtcttgttataattagcttcttggggtatctttaaatactgtagaaaagaggaaggaaataataaatggctaaaatgagaatatcaccggaattgaaaaaactgatcgaaaaataccgctgcgtaaaagatacggaaggaatgtctcctgctaaggtatataagctggtgggagaaaatgaaaacctatatttaaaaatgacggacagccggtataaagggaccacctatgatgtggaacgggaaaaggacatgatgctatggctggaaggaaagctgcctgttccaaaggtcctgcactttgaacggcatgatggctggagcaatctgctcatgagtgaggccgatggcgtcctttgctcggaagagtatgaagatgaacaaagccctgaaaagattatcgagctgtatgcggagtgcatcaggctctttcactccatcgacatatcggattgtccctatacgaatagcttagacagccgcttagccgaattggattacttactgaataacgatctggccgatgtggattgcgaaaactgggaagaagacactccatttaaagatccgcgcgagctgtatgattttttaaagacggaaaagcccgaagaggaacttgtcttttcccacggcgacctgggagacagcaacatctttgtgaaagatggcaaagtaagtggctttattgatcttgggagaagcggcagggcggacaagtggtatgacattgccttctgcgtccggtcgatcagggaggatatcggggaagaacagtatgtcgagctattttttgacttactggggatcaagcctgattgggagaaaataaaatattatattttactggatgaattgttttagtacctagatgtggcgcaacgatgccggcgacaagcaggagcgcaccgacttcttccgcatcaagtgttttggctctcaggccgaggcccacggcaagtatttgggcaaggggtcgctggtattcgtgcagggcaagattcggaataccaagtacgagaaggacggccagacggtctacgggaccgacttcattgccgataaggtggattatctggacaccaaggcaccaggcgggtcaaatcaggaataagggcacattgccccggcgtgagtcggggcaatcccgcaaggagggtgaatgaatcggacgtttgaccggaaggcatacaggcaagaactgatcgacgcggggttttccgccgaggatgccgaaaccatcgcaagccgcaccgtcatgcgtgcgccccgcgaaaccttccagtccgtcggctcgatggtccagcaagctacggccaagatcgagcgcgacagcgtgcaactggctccccctgccctgcccgcgccatcggccgccgtggagcgttcgcgtcgtctcgaacaggaggcggcaggtttggcgaagtcgatgaccatcgacacgcgaggaactatgacgaccaagaagcgaaaaaccgccggcgaggacctggcaaaacaggtcagcgaggccaagcaggccgcgttgctgaaacacacgaagcagcagatcaaggaaatgcagctttccttgttcgatattgcgccgtggccggacacgatgcgagcgatgccaaacgacacggcccgctctgccctgttcaccacgcgcaacaagaaaatcccgcgcgaggcgctgcaaaacaaggtcattttccacgtcaacaaggacgtgaagatcacctacaccggcgtcgagctgcgggccgacgatgacgaactggtgtggcagcaggtgttggagtacgcgaagcgcacccctatcggcgagccgatcaccttcacgttctacgagctttgccaggacctgggctggtcgatcaatggccggtattacacgaaggccgaggaatgcctgtcgcgcctacaggcgacggcgatgggcttcacgtccgaccgcgttgggcacctggaatcggtgtcgctgctgcaccgcttccgcgtcctggaccgtggcaagaaaacgtcccgttgccaggtcctgatcgacgaggaaatcgtcgtgctgtttgctggcgaccactacacgaaattcatatgggagaagtaccgcaagctgtcgccgacggcccgacggatgttcgactatttcagctcgcaccgggagccgtacccgctcaagctggaaaccttccgcctcatgtgcggatcggattccacccgcgtgaagaagtggcgcgagcaggtcggcgaagcctgcgaagagttgcgaggcagcggcctggtggaacacgcctgggtcaatgatgacctggtgcattgcaaacgctagggccttgtggggtcagttccggctgggggttcagccagcgctttactgagatctggggaaccctgtggttggcatgcacatacaaatggacgaacggataaaccttttcacgcccttttaaatatccgattattctaataaacgctcttttctcttaggtttacccgccaatatatcctgtcaaacactgatagtttaaactgaaggcgggaaacgacaatctgatcatgagcggagaattaagggagtcacgttatgacccccgccgatgacgcgggacaagccgttttacgtttggaactgacagaaccgcaacgttgaaggagccactcagccgcgggtttctggagtttaatgagctaagcacatacgtcagaaaccattattgcgcgttcaaaagtcgcctaaggtcactatcagctagcaaatatttcttgtcaaaaatgctccactgacgttccataaattcccctcggtatccaattagagtctcatattcactctcaatccaaataatctgcaccggatctggatcgtttcgcatgattgaacaagatggattgcacgcaggttctccggccgcttgggtggagaggctattcggctatgactgggcacaacagacaatcggctgctctgatgccgccgtgttccggctgtcagcgcaggggcgcccggttctttttgtcaagaccgacctgtccggtgccctgaatgaactgcaggacgaggcagcgcggctatcgtggctggccacgacgggcgttccttgcgcagctgtgctcgacgttgtcactgaagcgggaagggactggctgctattgggcgaagtgccggggcaggatctcctgtcatctcaccttgctcctgccgagaaagtatccatcatggctgatgcaatgcggcggctgcatacgcttgatccggctacctgcccattcgaccaccaagcgaaacatcgcatcgagcgagcacgtactcggatggaagccggtcttgtcgatcaggatgatctggacgaagagcatcaggggctcgcgccagccgaactgttcgccaggctcaaggcgcgcatgcccgacggcgatgatctcgtcgtgacccatggcgatgcctgcttgccgaatatcatggtggaaaatggccgcttttctggattcatcgactgtggccggctgggtgtggcggaccgctatcaggacatagcgttggctacccgtgatattgctgaagagcttggcggcgaatgggctgaccgcttcctcgtgctttacggtatcgccgctcccgattcgcagcgcatcgccttctatcgccttcttgacgagttcttctgagcgggactctggggttcgaaatgaccgaccaagcgacgcccaacctgccatcacgagatttcgattccaccgccgccttctatgaaaggttgggcttcggaatcgttttccgggacgccggctggatgatcctccagcgcggggatctcatgctggagttcttcgcccacgggatctctgcggaacaggcggtcgaaggtgccgatatcattacgacagcaacggccgacaagcacaacgccacgatcctgagcgacaatatgatcgggcccggcgtccacatcaacggcgtcggcggcgactgcccaggcaagaccgagatgcaccgcgatatcttgctgcgttcggatattttcgtggagttcccgccacagacccggatgatccccgatcgttcaaacatttggcaataaagtttcttaagattgaatcctgttgccggtcttgcgatgattatcatataatttctgttgaattacgttaagcatgtaataattaacatgtaatgcatgacgttatttatgagatgggtttttatgattagagtcccgcaattatacatttaatacgcgatagaaaacaaaatatagcgcgcaaactaggataaattatcgcgcgcggtgtcatctatgttactagatcgggccaatacgcaaaccgcctctccccgcgcgttggccgattcattaatgcagctggcacgacaggtttcccgactggaaagcgggcagtgagcgcaacgcaattaatgtgagttagctcactcattaggcaccccaggctttacactttatgcttccggctcgtatgttgtgtggaattgtgagcggataacaatttcacacaggaaacagctatgaccatgattacgccaagcttgagctcctgcaggtcactggattttggttttaggaattagaaattttattgatagaagtattttacaaatacaaatacatactaagggtttcttatatgctcaacacatgagcgaaaccctataagaaccctaattcccttatctgggaactactcacacattattctggagaaaatagagagagatagatttgtagagagagactggtgatttttgcggactctatcgacggatcgggctagagttcgtctttggaaccattcagatcctcttctgagatgagtttttgttctgcggccgcgtaacaagtcccgccggtatcggacataatgagggaaacattatacaatgtcggtttgctagcaacagaggcgtcaaaatgaaccggcacatagggatttccttcgcaggcgacaattatgtgtttattagcttgagtagttttataagcgcaatttggatatttgctagacccagtttctcggcaatcggtgatagacatggtggagtagctttggtagcaattcgtttgaccattcttacaagccacattcttttgtgaacaaacagcctgaacatctgccaatgactcgtggacaaatgtgtttacaggcttacacctgtcctttgtaaggttacgtgacttcatcatctggttacagtagttactagaactggatcctgctaaacatgtgcttgtaaagagaagcaaggaaagtgaaagcaaagatagaaaaggtttggaagccatggttcccggccgggtcagatcctctagagtcgatcgaggtcctctccaaatgaaatgaacttccttatatagaggaagggtcttgcgaaggatagtgggattgtgcgtcatcccttacgtcagtggagatatcacatcaatccacttgctttgaagacgtggttggaacgtcttctttttccacgatgttcctcgtgggtgggggtccatctttgggaccactgtcggtagaggcattcttgaacgatagcctttcctttatcgcaatgatggcatttgtagaagccatcttccttttctactgtcctttcgatgaagtgacagatagctgggcaatggaatccgaggaggtttcccgatattaccctttgttgaaaagtctcaatagccctctggtcttctgagactgtatctttgatattcttggagtagacgagagtgtcgtgctccaccatgttgacctgcaggtcgacaagcttatcgataccgtcgacctcgagggggggcccggtaccaaaaccaccccagtacattaaaaacgtccgcaatgtgttattaagttgtctaagcgtcaatttgtttacaccacaatatatcctgccaccagccagccaacagctccccgaccggcagctcggcacaaaatcaccactcgatacaggcagcccatcagtccactaga

SEQ ID NO: 30 - protein, 19 aa, Suncus murinus
KPTLYNVSLVLSDTASTCY

SEQ ID NO: 31 - protein, 19 aa, Bos taurus
KPTLYNVSLVLSDTASTCY

SEQ ID NO: 32 - protein, 19 aa, Trachemys scripta elegans
KPTAVNVSVILSDTDITCY

SEQ ID NO: 33 - protein, 19 aa, Mesocricetus auratus
KPTLYNVSLIMSDAGGTCY

SEQ ID NO: 34 - protein, 19 aa, Homo sapiens
KPTHVNVSVVMAEVDGTCY

SEQ ID NO: 35 - protein, 567 aa, Avian influenza virus
MEKIVLLFAIVSLVKSDQICIGYHANNSTEQVDTIMEKNVTVTHAQDILEKTHNGKLCDLDGVKPLILRDCSVAGWLLGNPMCDEFINVPEWSYIVEKANPVNDLCYPGDFNDYEELKHLLSRINHFEKIQIIPKSSWPSHEASLGVSSACPYQGKSSFFRNVVWLIKKNSTYPTIKRSYNNTNQEDLLVLWGIHHPNDAAEQTKLYQNPTTYISVGTSTLNQRLVPRIATRSKVNGQSGRMEFFWTILKPNDAINFESNGNFIAPEYAYKIVKKGDSTIMKSELEYGNCNTKCQTPMGAINSSMPFHNIHPLTIGECPKYVKSNRLVLATGLRNSPQRERRKKRGLFGAIAGFIEGGWQGMVDGWYGYHHSNEQGSGYAADKESTQKAIDGVTNKVNSIIDKMNTQFEAVGREFNNLERRIENLNKKMEDGFLDVWTYNAELLVLMENERTLDFHDSNVKNLYDKVRLQLRDNAKELGNGCFEFYHKCDNECMESVRNGTYDYPQYSEEAKLKREEISGVKLESIGIYQILTIYSTVASSLALAIMVAGLSLWMCSNGSLQCRICI

SEQ ID NO: 36 - protein, 567 aa, Avian Influenza virus
MEKIVLLFATISLVKSDHICIGYHANNSTEQVDTIMEKNVTVTHAQDILEKTHNGKLCDLNGVKPLILKDCSVAGWLLGNPLCDEFINVPEWSYIVEKPNPANDLCYPGNFNDYEELKHLLSRINHFEKIQIIPKDSWSNHEASLGVSAACSYQGNSSFFRNVVWLIKKDNAYPTIKKGYNNTNREDLLILWGIHHPNDEAEQTRLYQNPTTYISIGTSTLNQRLVPKIATRSKINGQSGRIDFFWTILKPNDAIHFESNGNFIAPEYAYKIVKKGDSTIMRSEVEYGNCNTRCQTPIGAINSSMPFHNIHPLTIGECPKYVKSNKLVLATGLRNSPQRERRRKRGLFGAIAGFIEGGWQGMVDGWYGYHHSNEQGSGYAADKESTQKAIDGVTNKVNSIIDKMNTQFEAVGREFNNLERRIENLNKKMEDGFLDVWTYNAELLVLMENERTLDFHDSNVKNLYDKVRLQLKDNAKELGNGCFEFYHKCNNECMESVRNGTYDYPQYSEEARLKREEISGVKLESIGIYQILSIYSTVASSLALAIMMAGLSLWMCSNGSLQCRICI

SEQ ID NO: 37 - protein, 238 aa, Artificial Sequence
  enhanced green fluorescent protein (eGFP)
VSKGEELFTGVVPILVELDGDVNGHKFSVSGEGEGDATYGKLTLKFICTTGKLPVPWPTLVTTLTYGVQCFSRYPDHMKQHDFFKSAMPEGYVQERTIFFKDDGNYKTRAEVKFEGDTLVNRIELKGIDFKEDGNILGHKLEYNYNSHNVYIMADKQKNGIKVNFKIRHNIEDGSVQLADHYQQNTPIGDGPVLLPDNHYLSTQSALSKDPNEKRDHMVLLEFVTAAGITLGMDELYK